European Patent Application EP 4 389 892 A1, published June 26, 2024. Title: Antisense oligonucleotide targeting CAV3.1 gene and use thereof. Applicant: Korea Advanced Insistitute of Science and Technology. Application KR. The sequence listing filed with the application follows.

SEQUENCE LISTING (64 sequences)

SEQ ID NO: 1 - DNA, 1660 bp, Homo sapiens
  source 1..1660: mol_type = genomic DNA
gggagagaggaggcatggtggacaacagaggtcaggctgcaatgacccctatctactagtaagagcggctaccaggacctctgcttaggatagtcctgctgtgcctggtggtggtgggcagggggcacagccagcttgacaggagggctagtccatgctggagaggagactgctgggctgagccctcccccaccccatataggcagcaataaggactgactccttggacgttcagggtctgggcagccgggaagacctgctggcagaggtgagtgggccctccccgcccctggcccgggcctactctttctggggccagtcaagtacccaggcacagcagcactcccgcagccacagcaagatctccaagcacatgaccccgccagccccttgcccaggcccagaacccaactggggcaagggccctccagagaccagaagcagcttagagttggacacggagctgagctggatttcaggagacctcctgccccctggcggccaggaggagcccccatccccacgggacctgaagaagtgctacagcgtggaggcccagagctgccagcgccggcctacgtcctggctggatgagcagaggagacactctatcgccgtcagctgcctggacagcggctcccaaccccacctgggcacagacccctctaaccttgggggccagcctcttggggggcctgggagccggcccaagaaaaaactcagcccgcctagtatcaccatagacccccccgagagccaaggtcctcggaccccgcccagccctggtatctgcctccggaggagggctccgtccagcgactccaaggatcccttggcctctggcccccctgacagcatggctgcctcgccctccccaaagaaagatgtgctgagtctctccggtttatcctctgacccagcagacctggacccctgagtcctgccccactttcccactcacctttctccactgggtgccaagtcctagctcctcctcctgggctatattcctgacaaaagttccatatagacaccaaggaggcggaggcgctcctccctgcctcagtggctctgggtacctgcaagcagaacttccaaagagagttaaaagcagcagccccggcaactctggctccaggcagaaggagaggcccggtgcagctgaggttcccgacaccagaagctgttgggagaaagcaatacgtttgtgcagaatctctatgtatattctattttattaaattaattgaatctagtatatgcgggatgtacgacattttgtgactgaagagacttgtttccttctacttttatgtgtctcagaatatttttgaggcgaaggcgtctgtctcttggctattttaacctaaaataacagtctagttatattccctcttcttgcaaagcacaagctgggaccgcgagcacattgcagccccaacggtggcccatcttcagcggagagcgagaaccattttggaaactgtaatgtaacttattttttcctttaacctcgtcatcattttctgtagggaaaaaaaaaagaaaaagaaaaaatgagattttacaagtgaaatggaacctttttatatatacatacatacatatctatctatctatctatatatatataaaataaagtaattttcctaaataaaaa

SEQ ID NO: 2 - DNA, 20 bp, synthetic construct
  misc_feature 1..20: note = CACNA1G_gapmer_73_ASO
  source 1..20: mol_type = other DNA
  misc_RNA 1..5: note = ribunucleotides but alll uracils are substituted with thymines.
  misc_RNA 16..20: note = ribonucleotides but all uracils are substituted with thymines.
tcaagtagaagaaaaccacc

SEQ ID NO: 3 - DNA, 20 bp, synthetic construct
  misc_feature 1..20: note = CACNA1G_gapmer_74_ASO
  misc_RNA 1..5: note = ribonucleotides but all uracils are substituted with thymines.
  source 1..20: mol_type = other DNA
  misc_RNA 16..20: note = ribonucleotides but all uracils are substituted with thymines.
gtcagtaaaaacctcagcct

SEQ ID NO: 4 - DNA, 20 bp, synthetic construct
  misc_feature 1..20: note = CACNA1G_gapmer_75_ASO
  misc_RNA 1..5: note = ribonucleotides but all uracils are substituted with thymines.
  source 1..20: mol_type = other DNA
  misc_RNA 16..20: note = ribonucleotides but all uracils are substituted with thymines.
atctccttgttgtgcctcca

SEQ ID NO: 5 - DNA, 20 bp, synthetic construct
  misc_feature 1..20: note = CACNA1G_gapmer_76_ASO
  misc_RNA 1..5: note = ribonucleotides but all uracils are substituted with thymines.
  source 1..20: mol_type = other DNA
  misc_RNA 16..20: note = ribonucleotides but all uracils are substituted with thymines.
ccaaatgagaaaaagctgtg

SEQ ID NO: 6 - DNA, 20 bp, synthetic construct
  misc_feature 1..20: note = CACNA1G_gapmer_77_ASO
  misc_RNA 1..5: note = ribonucleotides but all uracils are substituted with thymines.
  source 1..20: mol_type = other DNA
  misc_RNA 16..20: note = ribonucleotides but all uracils are substituted with thymines.
tgactatgagagacctgtgc

SEQ ID NO: 7 - DNA, 20 bp, synthetic construct
  misc_feature 1..20: note = CACNA1G_gapmer_78_ASO
  misc_RNA 1..5: note = ribonucleotides but all uracils are substituted with thymines.
  source 1..20: mol_type = other DNA
  misc_RNA 16..20: note = ribonucleotides but all uracils are substituted with thymines.
ctgtgtgatgttcttctgtt

SEQ ID NO: 8 - DNA, 20 bp, synthetic construct
  misc_feature 1..20: note = CACNA1G_gapmer_79_ASO
  misc_RNA 1..5: note = ribonucleotides but all uracils are substituted with thymines.
  source 1..20: mol_type = other DNA
  misc_RNA 16..20: note = ribonucleotides but all uracils are substituted with thymines.
catagccaatgttgtcaaag

SEQ ID NO: 9 - DNA, 20 bp, synthetic construct
  misc_feature 1..20: note = CACNA1G_gapmer_80_ASO
  misc_RNA 1..5: note = ribonucleotides but all uracils are substituted with thymines.
  source 1..20: mol_type = other DNA
  misc_RNA 16..20: note = ribonucleotides but all uracils are substituted with thymines.
ctagtgtgattccagagagc

SEQ ID NO: 10 - DNA, 20 bp, synthetic construct
  misc_feature 1..20: note = CACNA1G_gapmer_81_ASO
  misc_RNA 1..5: note = ribonucleotides but all uracils are substituted with thymines.
  source 1..20: mol_type = other DNA
  misc_RNA 16..20: note = ribonucleotides but all uracils are substituted with thymines.
tacctgatgaccacaatgac

SEQ ID NO: 11 - DNA, 20 bp, synthetic construct
  misc_feature 1..20: note = CACNA1G_gapmer_82_ASO
  misc_RNA 1..5: note = ribonucleotides but all uracils are substituted with thymines.
  source 1..20: mol_type = other DNA
  misc_RNA 16..20: note = ribonucleotides but all uracils are substituted with thymines.
tacttgattgctacttttga

SEQ ID NO: 12 - DNA, 20 bp, synthetic construct
  misc_feature 1..20: note = CACNA1G_gapmer_83_ASO
  misc_RNA 1..5: note = ribonucleotides but all uracils are substituted with thymines.
  source 1..20: mol_type = other DNA
  misc_RNA 16..20: note = ribonucleotides but all uracils are substituted with thymines.
tggttccagttgacacaggt

SEQ ID NO: 13 - DNA, 20 bp, synthetic construct
  misc_feature 1..20: note = CACNA1G_gapmer_84_ASO
  misc_RNA 1..5: note = ribonucleotides but all uracils are substituted with thymines.
  source 1..20: mol_type = other DNA
  misc_RNA 16..20: note = ribonucleotides but all uracils are substituted with thymines.
ccattggcatccctgtcctg

SEQ ID NO: 14 - DNA, 20 bp, synthetic construct
  misc_feature 1..20: note = CACNA1G_gapmer_85_ASO
  misc_RNA 1..5: note = ribonucleotides but all uracils are substituted with thymines
  source 1..20: mol_type = other DNA
  misc_RNA 16..20: note = ribonucleotides but all uracils are substituted with thymines
tacagcttaactgtccactc

SEQ ID NO: 15 - DNA, 20 bp, synthetic construct
  misc_feature 1..20: note = CACNA1G_gapmer_86_ASO
  mat_peptide 1..5: note = ribonucleotides but all uracils are substituted with thymines
  source 1..20: mol_type = other DNA
  misc_RNA 16..20: note = ribonucleotides but all uracils are substituted with thymines
ttcttagcaggtcagtaggt

SEQ ID NO: 16 - DNA, 20 bp, synthetic construct
  misc_feature 1..20: note = CACNA1G_gapmer_87_ASO
  misc_RNA 1..5: note = nibonucleotides but all uracils are substituted with thymines.
  source 1..20: mol_type = other DNA
  misc_RNA 16..20: note = ribonucleotides but all uracils are substituted with thymines.
accttcactgtcatttcagc

SEQ ID NO: 17 - DNA, 20 bp, synthetic construct
  misc_feature 1..20: note = CACNA1G_gapmer_88_ASO
  source 1..20: mol_type = other DNA
  misc_RNA 1..5: note = ribonucleotides but all uracils are substituted with thymines.
  misc_RNA 16..20: note = ribonucleotides but all uracils are substituted with thymines.
ggagattggaaattggacat

SEQ ID NO: 18 - DNA, 20 bp, synthetic construct
  misc_feature 1..20: note = CACNA1G_gapmer_89_ASO
  misc_RNA 1..5: note = ribonucleotides but all uracils are substituted with thymines.
  source 1..20: mol_type = other DNA
  misc_RNA 16..20: note = ribonucleotides but all uracils are substituted with thymines.
gtgttgtagcaggtggactc

SEQ ID NO: 19 - DNA, 20 bp, synthetic construct
  misc_feature 1..20: note = CACNA1G_gapmer_90_ASO
  misc_RNA 1..5: note = ribonucleotides but all uracils are substituted with thymines.
  source 1..20: mol_type = other DNA
  misc_RNA 16..20: note = ribonucleotides but all uracils are substituted with thymines.
tcatcaggcaaagagtcatc

SEQ ID NO: 20 - DNA, 20 bp, synthetic construct
  misc_feature 1..20: note = CACNA1G_gapmer_91_ASO
  misc_RNA 1..5: note = ribonucleotides but all uracils are substituted with thymines.
  source 1..20: mol_type = other DNA
  misc_RNA 16..20: note = ribonucleotides but all uracils are substituted with thymines.
gtcagtccttattgctgcct

SEQ ID NO: 21 - DNA, 20 bp, synthetic construct
  misc_feature 1..20: note = CACNA1G_gapmer_92_ASO
  misc_RNA 1..5: note = ribonucleotides but all uracils are substituted with thymines.
  source 1..20: mol_type = other DNA
  misc_RNA 16..20: note = ribonucleotides but all uracils are substituted with thymines.
tattgctttctcccaacagc

SEQ ID NO: 22 - DNA, 20 bp, synthetic construct
  misc_feature 1..20: note = sh3.1_20mer
  misc_RNA 1..5: note = ribonucleotides but all uracils are substituted with thymines.
  source 1..20: mol_type = other DNA
  misc_RNA 16..20: note = ribonucleotides but all uracils are substituted with thymines.
acttgctgtccacaatcttt

SEQ ID NO: 23 - DNA, 20 bp, synthetic construct
  misc_feature 1..20: note = AS-CAv3.1_20mer
  misc_RNA 1..5: note = ribonucleotides but all uracils are substituted with thymines.
  source 1..20: mol_type = other DNA
  misc_RNA 16..20: note = ribonucleotides but all uracils are substituted with thymines.
cgggacccattggcatccct

SEQ ID NO: 24 - DNA, 20 bp, synthetic construct
  misc_feature 1..20: note = scrambled
  misc_RNA 1..5: note = ribonucleotides but all uracils are substituted with thymines.
  source 1..20: mol_type = other DNA
  misc_RNA 16..20: note = ribonucleotides but all uracils are substituted with thymines.
cctataggactatccaggaa

SEQ ID NO: 25 - DNA, 20 bp, synthetic construct
  misc_feature 1..20: note = HTTRX_ASO
  misc_RNA 1..5: note = ribonucleotides but all uracils are substituted with thymines.
  source 1..20: mol_type = other DNA
  misc_RNA 16..20: note = ribonucleotides but all uracils are substituted with thymines.
ctcagtaacattgacaccac

SEQ ID NO: 26 - DNA, 20 bp, Homo sapiens
  misc_feature 1..20: note = CACNA1G_gapmer_73_target
  source 1..20: mol_type = genomic DNA
ggtggttttcttctacttga

SEQ ID NO: 27 - DNA, 20 bp, Homo sapiens
  misc_feature 1..20: note = CACNA1G_gapmer_74_target
  source 1..20: mol_type = genomic DNA
aggctgaggtttttactgac

SEQ ID NO: 28 - DNA, 20 bp, Homo sapiens
  misc_feature 1..20: note = CACNA1G_gapmer_75_target
  source 1..20: mol_type = genomic DNA
tggaggcacaacaaggagat

SEQ ID NO: 29 - DNA, 20 bp, Homo sapiens
  misc_feature 1..20: note = CACNA1G_gapmer_76_target
  source 1..20: mol_type = genomic DNA
cacagctttttctcatttgg

SEQ ID NO: 30 - DNA, 20 bp, Homo sapiens
  misc_feature 1..20: note = CACNA1G_gapmer_77_target
  source 1..20: mol_type = genomic DNA
tggaggcacaacaaggagat

SEQ ID NO: 31 - DNA, 20 bp, Homo sapiens
  misc_feature 1..20: note = CACNA1G_gapmer_78_target
  source 1..20: mol_type = genomic DNA
aacagaagaacatcacacag

SEQ ID NO: 32 - DNA, 20 bp, Homo sapiens
  misc_feature 1..20: note = CACNA1G_gapmer_79_target
  source 1..20: mol_type = genomic DNA
ctttgacaacattggctatg

SEQ ID NO: 33 - DNA, 20 bp, Homo sapiens
  misc_feature 1..20: note = CACNA1G_gapmer_80_target
  source 1..20: mol_type = genomic DNA
gctctctggaatcacactag

SEQ ID NO: 34 - DNA, 20 bp, Homo sapiens
  source 1..20: mol_type = genomic DNA
  misc_feature 1..20: note = CACNA1G_gapmer_81_target
gtcattgtggtcatcaggta

SEQ ID NO: 35 - DNA, 20 bp, Homo sapiens
  misc_feature 1..20: note = CACNA1G_gapmer_82_target
  source 1..20: mol_type = genomic DNA
tcaaaagtagcaatcaagta

SEQ ID NO: 36 - DNA, 20 bp, Homo sapiens
  misc_feature 1..20: note = CACNA1G_gapmer_83_target
  source 1..20: mol_type = genomic DNA
acctgtgtcaactggaacca

SEQ ID NO: 37 - DNA, 20 bp, Homo sapiens
  misc_feature 1..20: note = CACNA1G_gapmer_84_target
  source 1..20: mol_type = genomic DNA
caggacagggatgccaatgg

SEQ ID NO: 38 - DNA, 20 bp, Homo sapiens
  misc_feature 1..20: note = CACNA1G_gapmer_85_target
  source 1..20: mol_type = genomic DNA
gagtggacagttaagctgta

SEQ ID NO: 39 - DNA, 20 bp, Homo sapiens
  misc_feature 1..20: note = CACNA1G_gapmer_86_target
  source 1..20: mol_type = genomic DNA
acctactgacctgctaagaa

SEQ ID NO: 40 - DNA, 20 bp, Homo sapiens
  misc_feature 1..20: note = CACNA1G_gapmer_87_target
  source 1..20: mol_type = genomic DNA
gctgaaatgacagtgaaggt

SEQ ID NO: 41 - DNA, 20 bp, Homo sapiens
  misc_feature 1..20: note = CACNA1G_gapmer_88_target
  source 1..20: mol_type = genomic DNA
atgtccaatttccaatctcc

SEQ ID NO: 42 - DNA, 20 bp, Homo sapiens
  misc_feature 1..20: note = CACNA1G_gapmer_89_target
  source 1..20: mol_type = genomic DNA
gagtccacctgctacaacac

SEQ ID NO: 43 - DNA, 20 bp, Homo sapiens
  misc_feature 1..20: note = CACNA1G_gapmer_90_target
  source 1..20: mol_type = genomic DNA
gatgactctttgcctgatga

SEQ ID NO: 44 - DNA, 20 bp, Homo sapiens
  misc_feature 1..20: note = CACNA1G_gapmer_91_target
  source 1..20: mol_type = genomic DNA
aggcagcaataaggactgac

SEQ ID NO: 45 - DNA, 20 bp, Homo sapiens
  misc_feature 1..20: note = CACNA1G_gapmer_92_target
  source 1..20: mol_type = genomic DNA
gctgttgggagaaagcaata

SEQ ID NO: 46 - DNA, 20 bp, Homo sapiens
  misc_feature 1..20: note = sh3.1_20mer_target
  source 1..20: mol_type = genomic DNA
aaagattgtggacagcaagt

SEQ ID NO: 47 - DNA, 20 bp, Homo sapiens
  misc_feature 1..20: note = AS-CAv3.1_20mer_target
  source 1..20: mol_type = genomic DNA
agggatgccaatgggtcccg

SEQ ID NO: 48 - DNA, 20 bp, synthetic construct
  misc_feature 1..20: note = scrambled_target
  source 1..20: mol_type = other DNA
ttcctggatagtcctatagg

SEQ ID NO: 49 - DNA, 20 bp, Homo sapiens
  misc_feature 1..20: note = HTTRX_target
  source 1..20: mol_type = genomic DNA
gtggtgtcaatgttactgag

SEQ ID NO: 50 - DNA, 24 bp, synthetic construct
  misc_feature 1..24: note = Cav3.1 probe
  source 1..24: mol_type = other DNA
tgtcattgggcagagagtgtgtcc

SEQ ID NO: 51 - DNA, 20 bp, synthetic construct
  misc_feature 1..20: note = Cav3.1 qPCR-F
  source 1..20: mol_type = other DNA
gaggaagtctggtgtcagcc

SEQ ID NO: 52 - DNA, 20 bp, synthetic construct
  misc_feature 1..20: note = Cav3.1 qPCR-R
  source 1..20: mol_type = other DNA
tgtcctagggatctctcggc

SEQ ID NO: 53 - DNA, 27 bp, synthetic construct
  misc_feature 1..27: note = Cav3.2 probe
  source 1..27: mol_type = other DNA
accttggtcttcttttcatgctcctgt

SEQ ID NO: 54 - DNA, 20 bp, synthetic construct
  misc_feature 1..20: note = Cav3.2 qPCR-F
  source 1..20: mol_type = other DNA
gacactgtggttcaagctct

SEQ ID NO: 55 - DNA, 21 bp, synthetic construct
  misc_feature 1..21: note = Cav3.2 qPCR-R
  source 1..21: mol_type = other DNA
ttatcctcgctgcattctagc

SEQ ID NO: 56 - DNA, 24 bp, synthetic construct
  misc_feature 1..24: note = Cav3.3 probe
  source 1..24: mol_type = other DNA
acactgtgtcctcagagcaagcag

SEQ ID NO: 57 - DNA, 20 bp, synthetic construct
  misc_feature 1..20: note = Cav3.3 qPCR-F
  source 1..20: mol_type = other DNA
gggagggatgttcaggcatc

SEQ ID NO: 58 - DNA, 20 bp, synthetic construct
  misc_feature 1..20: note = Cav3.3 qPCR-R
  source 1..20: mol_type = other DNA
gagcttccttcatccccacc

SEQ ID NO: 59 - DNA, 20 bp, Homo sapiens
  source 1..20: mol_type = genomic DNA
  misc_feature 1..20: note = Target sequence of CACNA1G_gapmer_4_ASO
tggacacggagctgagctgg

SEQ ID NO: 60 - DNA, 20 bp, Homo sapiens
  source 1..20: mol_type = genomic DNA
  misc_feature 1..20: note = Target sequence of CACNA_gapmer_7_ASO
gaaagcaatacgtttgtgca

SEQ ID NO: 61 - DNA, 20 bp, Homo sapiens
  source 1..20: mol_type = genomic DNA
  misc_feature 1..20: note = Target sequence of CACNA1G_gapmer_11_ASO
gacattttgtgactgaagag

SEQ ID NO: 62 - DNA, 20 bp, synthetic construct
  misc_RNA 1..5: note = All uracils are substituted with thymines.
  source 1..20: mol_type = other DNA
  misc_RNA 16..20: note = All uracils are substituted with thymines.
  misc_feature 1..20: note = CACNA1G_gapmer_4_ASO
ccagctcagctccgtgtcca

SEQ ID NO: 63 - DNA, 20 bp, synthetic construct
  source 1..20: mol_type = other DNA
  misc_RNA 1..5: note = ribonucleotides but all uracils are substituted with thymines.
  misc_RNA 16..20: note = ribonucleotides but all uracils are substituted with thymines.
  misc_feature 1..20: note = CACNA1G_gapmer_7_ASO
tgcacaaacgtattgctttc

SEQ ID NO: 64 - DNA, 20 bp, synthetic construct
  source 1..20: mol_type = other DNA
  misc_RNA 1..5: note = all uracils are substituted with thymines.
  misc_RNA 16..20: note = all uracils are substituted with thymines.
  misc_feature 1..20: note = CACNA1G_gapmer_11_ASO
ctcttcagtcacaaaatgtc